European Patent Application EP 4 299 746 A1, published January 3, 2024. Title: MODIFIED PRP43 HELICASE AND USE THEREOF. Applicant: Qitan Technology Ltd., Chengdu. The sequence listing filed with the application follows.

SEQUENCE LISTING (44 sequences)

SEQ ID NO: 1 - protein, 764 aa, Chaetomium thermophilum
  ctPrp43
MADITKGTKRLSGEAEGSQDSKRVKTNGDKMDAKNPYLAHLEEKPEADFESLLDKLERRNTTAKQAEAVEDSDINPWTGQRHSERYFKILKARRKLPVNKQRQEFLDLYHNNQILVFVGETGSGKTTQIPQYVLYDELPHQTGKLIACTQPRRVAAMSVAQRVADELDVKLGEEVGYSIRFENKTSSKTLLKYMTDGQLLREAMHDRDMSRYSCIILDEAHERTLATDILMALLKQLSERRKDLKIIVMSATLDAQKFQSYFFNAPLLAVPGRTHPVEIFYTPEAERDYVEAAIRTVLQIHACEPEGDILLFLTGEEEIEDACRRISLEVDEMIRESDAGPMSVYPLYGTLPPHQQQRIFEKAPQPFRPGGRPGRKCIVATNIAETSLTIDGIVYVVDPGFSKQKIYNPRTRVESLLVSPISKASAQQRAGRAGRTRPGKCFRLYTEEAFKKELIEQTYPEILRSNLSNTVLELKKLGVEDLVHFDLMDPPAPETMMRALEELNYLACLDDDGELTPLGNLASEFPLDPALAVMLISSPEFYCSNEILSITSLLSVPQIWVRPANARKRADEMKAQFAHPDGDHLTLLNAYHAYKGAEARGEDMKKWCHEHFLSYRHLSSADNVRAQLKKIMETHGIELVSTPFHDKNYYTNIRRALLAGFFMQVAMRESSNSKVYKTVKDEQLVLIHPSTTVTTPYEWVVYNEFVLTTKQYVRTVTNIRPEWLLEIAPVYYDLSTFQKGEIKNALTRVAEKIRRQQAMKASKA

SEQ ID NO: 2 - protein, 711 aa, Bathycoccus prasinos
  bpPrp43
MSSTTPKKKQRVQVSLDGDDANNKEEMMMINPYTHQPYSQTYLNILETRRKLPVWKQKSDFLHQLAASQTLVLVGETGSGKTTQIPQFLVDAGYTNEESKMVVCTQPRRVAAMSVAKRVAEEMDVQIGEEVGYSIRFEECTSRKTIMKYATDGMLLREAMTDPLLSRYSVIVIDEAHERTLATDVLFGLLKEVLKKRPEDLKCVVMSATLEAKKFQGYFEGAPLVMVPGRTHPVEIFYTQEPERDYLEAAIRTVVQIHRCEPPGDVLLFLTGEEEIEDACGKIRNEIKNIGDSVGPVNVVPLYSTLPPNQQQRIFDKAPDALTVGGVAGRKVVVSTNIAETSLTIDGIVYVVDPGFSKQKVYNPRSRVESLLVSPISRASAQQRAGRAGRTQPGKCFRLYTELSFKKDLIEQTYPEILRSNLGSVVIQLKKLGIDDLVHFDFMDPPAPETLMRALELLNYLGALDDEGELTKAGKIMSDFPLDPQLAKMLVGSTKFKCSNEIVTIVAMLSVPQCFIRPRDDQQRADAAKAHFAHLDGDHLTMLNAYHAFKQNGESQNWCWENYLNHRSLKSADNVRNQLVRLCQRHGVLLESTDFHSKDYYVNIRKAILNGFFMQVAHKERNGSYLTVKDNESVLLHPSTNLSGKPEWVVYNEFVLTSKKYVRTVTEIKGEWLIDLAEHYYDLSNFPSCAAKNALQQLYTQRERTHKGGKK

SEQ ID NO: 3 - protein, 533 aa, Uncultured bacterium
  unPrp43
MAVFSRKGSRVVKESRQQRERQRQAQEATNMAGTTLGNIMGAKEEDGDSALPIAGEEEAAKGGNKGNKFSEHMKKSTGASSFSQSKSLREQREFLPAFAVREELLRVIRENQVTIVIGETGSGKTTQLTQFLMEDGYGRAGMIGCTQPRRVAAMSVAKRVAEEMEVELGSAVGYSIRFEDVTSKETIIKYMTDGVLLRESLNEPDLDRYSCIIMDEAHERALNTDILMGLFKKVLQRRRDLKLIVTSATMNAKRFSDFYGGAPEFTIPGRTFPVDVMFHRSPVEDYVDGAVQQVLAIHVSMGPGDILVFMTGQEDIEVTCEQVQKRLDALNDPPKLSILPIYSQMPADLQAKIFDRAAPGVRKCIVATNIAETSLTVDGIKYVVDAGYSKMKVYNPKMGMDTLQITPISQANGSQRSGRAGRTGPGKAFRLYTEKAFKEELYLQTIPEIQRTNLANTVLMLKSLGVKDLLDFDFMDPPPQDTILTSMFDLWALGALDNLGELTGLGQKMSAFPMDPSLSKLLITAEEYGCSEE

SEQ ID NO: 4 - protein, 635 aa, Viral metagenome
  vmPrp43
MYSQKYYEILKKRQELPVWNSKNEFMEKLNNNECLVFVGETGSGKTTQIPQWCLEWSKTTRLAGKSLKVVCTQPRRVAAMSIATRVSEEMDVKLGDEVGYSIRFENCTSDKTVLQFSTDGMILLELTNDKILSKYSVIIIDEAHERTLSTDILMGMLKMILKIRTGDNGIKIVIMSATLDSEKFINYFDKCPLIEVPGRPHSIEIFYVKKQNIKYLEEAVLAVIQTHINEVEGDILLFLTGQEDIEEACKRIDEEKKKYSCRELTCIPLYSALSPSRQRLIFEPSRGRKCIVSTNIAETSLTIDGVIYVIDAGYSKLNVYNPILRIESLLITPITKASAKQRAGRAGRTSPGKVFRLYTEDIYHSVLPDQNIPEILRSNISTVVMQLKKFGIDDLVHFDFIDPPAPESLMRAIELLNYLGAIDDNCNLTSVGKMMVEFPLDPQLSKMIIASCDLKCSNEILSLASMLSVPSCFIGYNAKDKFAHKSGDHITLLNVYQAFKLNHEDIRWCNEYFISYRSLKSVDDVRRQLVQIMIKLNLNLVSAPNGEYTNIKKALVAGFFTQVANTVKIDKSRGHYLTFKDNQIAYVHPSSVLNRSPKWIIYNEYILTTRQYLRTVTEIEPDLLLQVEPKYFNNI

SEQ ID NO: 5 - protein, 628 aa, Archaeon
  arPrp43
MHCLFESYYCLYKFNVETGSGKSTQLPLYLHEGGWTKHGYSVVCTQPRRIAAITVASRVAEEFGCKLGEEVGYGIRFDFNCSDKTLIKYYTDGVLLRETMTDPLLQKYGVIIIDEAHQRTLHSDILMGLLKKIKKKRSDLRIIVTSATMDASAFKNFFELNDTNDRSQDTAVIMSVQGRQHLVDVLYVLESCRNYLSAAVDTVLSIHQYEDVGDILVFLPGGEEIDTAIAMLNERYEGNNMFFLPLYASLPHHMQMQVFQPTPPNMRKVVLATNIAEASITIEGIRYVVDSGYVKLNYIDVRSGLDALLCVPVTKSQAIQRAGRAGRTQPGKCFRLMTENTFISLDTNPPAEMQRVDISWAVLQLKALGIHDVLHFDFLSPPSSDSMIFALELLYSLGAIDDCCSITDLGAKMAEMPLEPRVAKCLLSSFDHGCCEEMLTIAAMVTVEYPFISQRRQASQESKVKLQKDMEHFAILGSDHLTLLRIYQEFTESNYAASWCDSMSLQFRILSRAKEIRYNLTNMLKRFKNEGDVLSSCGQDDKAVRRCLVSGFFSQAARLLADGKYHTLRGDVKVDAHPQSVVEQFGAPAEWVIYHEVIHSKATYIREISKIDPMWLHELAQHYYNLQM

SEQ ID NO: 6 - protein, 740 aa, Parcubacteria group bacterium GW2011
  paPrp43
MITTGELPILKHREEILESVIDHQVTVVIGETGSGKTTQIPQFLFELGSGLSGKIGVTQPRRVAATSVAYFVSRQLGCDIGQEVGYKIRFDDNTTEGTAIKFMTDGILLREMQSDPMLSEYSVIMVDEAHERSLNMDFLLGLLKGLLKKRSDLRLIVSSATIEEVKFSRYFSGAPVINVSGRTHPVDIKYCAGSGNLFPNTRDQTVELVEQIHRSTETGDILIFLDGEGAINGMIEEIERKQLPDLICLPLYGNMVFDEQMKVFKPTRERKVIVATNIAETSITIDGVVYVIDMGFEKRTGFHPETGIQSLDLSPISKASAAQRAGRAGRTQPGMCYRLYPENDFNSREEYTVPEIQRTDLAGVVLQMKSLGITDIENFDFIDPPDRESFEAAYKTLVILGALDKGNGLTSVGRLMAKLPLEPRIGRMLVAAQEYGCVDEVCIIAASLSSIRSVFARPKDKQFEADQAHKVFKDKTSDFLTLLSVYDAYERFGCDEQWCYQHFLNNRVLCEIRNVKNQLKDILSRAGISGSTKDPEKISKAVATGLVENIFQNLGHHAFGGSDGKFVYIHPGSVLFGEYALWMVAASIVETTKTFTRNCAVIEPSWIAEIAPQLCNTRTEANYSNQREGKIEAIKHIYFRDTEIKAESIWITVDEFKKIQEKKIVKAEAKGWLRLVFTKEPEKQSWENRNRWIAKVGDAVYEDDSYSSEPTRGRQYYCSPGHEFLGRIKVHREFEVMKFN

SEQ ID NO: 7 - protein, 1230 aa, Sorangium cellulosum
  scHrpA
GSPVRFPEELPISARVLDIARAIEAHQVVIVAGETGSGKTTQLPKICLAMGRGLSARIGVTQPRRIAATSVAARVAKELGVELGKEVGYKIRFSDRTSPATYVKYMTDGIVLAEIQGDPRLSDYDTLIIDEAHERSLNIDFLLGYLKRLLPRRPDLRVIVSSATLETDRFSSYFGGAPVIEVSGRTYPVEVIHRTPESGEAEVADAVANTVEEITSIDPRGDILVFLPGEREIHDTMAELERHGLPHTTLLPLYGRLPQGDQQRVFQPLPGRRIVLATNVAETSLTIPGIVYVVDAGLARVNRYSPRTGVTQLQIEPISRASADQRKGRAGRVQSGVCFRLYAEQDYQARPAYTDPEILRVGLSGVILQMKALGLGDIEDFPFLDAPSKRAVDEGYRVLEEIGALDDAGALTDIGRKLARLPLDPRLGRMVLGGEQEGALAEVLIIAAALGVQDPRERPLSAQKQADDAHRRFKDEGSDFAGLLKLWAFYQEAQGRLTQNQLRKTCRDHFISYLRMREWIDVHRQLSRITKDMGFSPNTTPAKGDAIHRALLPGLLSRIGMWNQENKVYLGARQTRFQLHPSSGLAKKPPAWIMAAELVETSQLFARMAAAVDPAWMEAAAGPLCKRSYGDPHWAAKPAAVMAKEQVTLYGLPIARDRRVDYGPIGPEPARRIFLLHALVRQEYATRAPFMDANRRLFEEVSRLRDKARRSEMLADEHALELFFDRRVPEGVYSGKTFEAWRKEAEAKDPRVLHLSIADVLLDEAAELSPERFPDALELYGATVPLSYRFDPGEDDDGIALALPLVLLPQADPDELEWMIPGWHAEKIALLLESLPKALRKALVPLREVAREIAADLRPFQGPMRAALARAVEDRTGERVPDDAFRPDELPPYLRFYFRVIGEDGRVIGEGRDLRELKDRLSGRARDAWAKVGKAGLERDGLTSFSLESLPERVQVDAGGQKVFGYPALIDGETSVSVRVLASRAAAAEATRAGLRRLLLLQLGSKMSQLEQPLRSAVAVSGLGAKVAPGEPGLARQIALRALDEAFQLGDPAAFPRTRAAFQARLDDGRRSLQAVLNRLAGLAREIGIELDRVQAMLRSMTGKPGASRPALDDARTQVELLLPVGLFSRAPLDRLAHLPRYLRAVQIRLERLPNGPQKDQTKAAQVLPFWQDYLKHQQGLRDKGVPAEDLESFRWLIEELRVSLFAPELKAAVPVSTQRLSEQWKRMMG

SEQ ID NO: 8 - protein, 767 aa, Candidatus Sungbacteria bacterium
  csHrpA
MELPILKERDRIIQAVSDNPVIVVVGETGSGKTTQIPIFLYEAGFAESGVIGITEPRRVAATSTAKYVAGVIGSTPGDLVGYQVRFDDETTVGTALKFMTDGILLREFQIDSNLSRYSVVLIDEAHERSQNVDFILGLLKDLLKRRRDLKVVVASATIDEQKFSNFFNRAPVINVSGRMFPVEVVWGKEDVDEEMIVEVMADAIAEIHRSEPEGDILSFMTGEDQIRRVVESLERMKLTDLVLVPAHASLPWEEQQKIFASYPGKRKVIVATNIAETSITIDGIVYVVDSGFIKQMNFHPESGIQSLDVVLHSKSGCEQRRGRAGRTQPGKCFRLYAESDFRERPQFTEPEIKRISLAGVVLAMKDIGIDKVEEFEFVDPPSREAFHEAHETLIALGAIQRGSHGLTDIGKMMAGLPLEPRIARMIIEAEKHGCTKDVATIAAFLSGRQVFARPKGKEIQADRAHVALKNPASDALTFLRVWDKYEDSDFDNQWCYDNFLNARVLREVDDIRYQLFNILESYGFEPTESSDTAVIAKAVAMGLAYSLLEHRSRHSYGGVLRQIDDVFIHPGSAIFGLSNSRWIVASEVVRTTKTYARGCTEVKPEWLPDMAPQHFKRGEPVVARYLKGAESAVISKAVLDGYGHELGSSEESVPVAEAIAIQKARVRDAESKGLLKLTFHNEASGRYSFTASFVAEAGGKRYKASYHAKVEEGVPYYCKVVDTYLGQTTVEPVFQVFAFNNPAPSPGQPLSSVEELAQKRGASLGRQ

SEQ ID NO: 9 - protein, 1311 aa, Mycolicibacterium chitae
  mcHrpA
MSDPSREAVRELRARLDDLTIRDAARLGRRLKGLRNPTPDALHKIENQIATGAALVTARRDAVPEISYPDLPVSASRDELAAAIAAHQVVVVAGATGSGKTTQLPKLCLELGRGIRGTIGHTQPRRLAARTVAQRIADELGTPLGETVGYTVRFTDQAGDRTLIKLMTDGILLAEIQRDRRLLRYDTLILDEAHERSLNIDFLLGYLRELLPRRPDLKVIVTSATIEPERFAAHFSGAPIVEVSGRTYPVEIRYRPLEVAVGGDAEDAVDPDDPDHDIVRTEVRDQTEAILDAVRELAAEPPGDVLVFLSGEREIRDTAEALRAADTGTRDLEVLPLYARLPTAEQQRVFAPRPASNLSRRIVLATNVAETSLTVPGIRYVVDPGSARISRYSRRTKVQRLPIEPISQASADQRAGRSGRTAPGVCIRLYSEPDFAARPRYTDPEILRTNLSAVILQMAALGLGDIESFPFLDPPDQRSIRDGVQLLQELGAFDARGAITDLGRRLAQLPVDPRLGRMILAADEQGCVEEVLVLAAALSIPDPRERPADREEAARQKHARFADENSDFVTYLNLWNYLGEQRKARSGNAFRRMCREEFLHYLRIREWQDLVGQLRSIAAGLGIRAGENAGAATDPNRVHAALIAGLLSHIGMREGDSREYQGARNSRFMLAPGSVLTKRPPRWLVVAELVETSRLYGRIAARIDPDTVEAIAGNLVQRSYSEPHWSAKRGAAMAYERVTLYGLPLVVRRQVDYARTDPELAREMFLRHALVDGEWQTRHHFFRDNAALRHELAEMEERARRRDLMVTDEEIYALYDARVPADIVSVRHFDAWWKKQRHRTPQLLTFTREELLRSDDADEHPDVWKADDVALPLTYRFEPGAEDDGVTVHVPLEVLARLGGDTFAWQVPALREELVTALIKSLPKDLRRNFVPAPDTARAVLPELAPEGEPLLDALQRALRRRTGVVVPISAFDLEKIPAHLRMTFAVENAEGAEVARGKDIDALRENLAGTTRAAVARAVADGVERTGLRDWPADLETLPKTVESVSGGNPVRGYPALVAAGPAVDVRVFSTPEEQRAAMREGTRALLRLVVPVPIKALERELDPRSRLILGNNPNGSLTALIEDCADAAIAALVPEPAWTRDDFAALRKQVAAGLGSRTRDLLARVQRVLAAYHDVRVALPDQPNAAQADAVADIRTQLADLMPAGFVSAAGAGHLGDLTRYLTAIARRLERLPQAPAADRERMLRVHTVEDAYHDLLQALSPVRAQAPEVREIGRQIEEFRVSLWAQQLGTPKPVSEQRIYRAIDAVLR

SEQ ID NO: 10 - protein, 1305 aa, Parcubacteria group bacterium ADurb.Bin305
  paHrpB
MAVENFDSQQYQNKSFSKAEQERDLELPILAYKKEIQEMISQNPTSIIVGETGSGKTTRIPLFLLETLEPDKKIAITQPRRVAARSVARFVADQVHCQVGEDVGYQVRFDDHTTEGTRINFMTDGILLRKIQEDQLLLDYEAVMVDEAHERSLNIDFALGLLKQLQKKRLEANVKPLKIIVSSATLEKEKFASYFSASPLLEVPGRLYPVDIHYEAERPRDYTEAAANKVAEIIGRTETGDILIFMPGQEEIDKTIKEIEKLKLQGVIILSLYGQMSAEEQDRIFEKTSARKIVVATNIAETSVTVPGIKYIIDSGLIKQTEFDPQSGIESLVVKPHAKSGCIQRAGRAGRLGPGECYRLYTEEDFYMRPEFQVPEIKRSNLAHVVLLMKQMGIEDVKSFDFIDPPDSESFKQALETLKTLGALDDDEKITKTGEVMAELPLEPHISRMVIEAQKHNCVETICTIAAFLGNKSVFVRPKEKTEEADEAHRKFKIPTSDFLTLLKVWEDYEAHDYNDTWARENFLNSKVLREVQNIRYQLFRVLHRNGIRATESRDEDAIGKSIAAGLVENLLEYNSRHAYQRIKDGSWGFYIHPSSVTFGEDPQFIVAAEIVSTNKTYARVNQQVKREWLKEIAPQFISEAPRSIYYDEEADKVIQEVSLYLKQTRSIVDLEKRQVTGEQAVEVFVEALMENNIDYPLLEKNLKVVELINKAWLKSGGKLDKEMSNIFTRNDLKEFYKTQLHGISSKQEMFKAIQEGKINLELNINEYVSPEHLEEILRNNPDTITLDGKEYQVAYEYDNQKKEPRASITMLVKDVLNFQEVPQLPSGRLLTLKVLEQEDSSKVLFESDNISEARQKARVFLINKQWKAWRESQDYESRIIRLENFNPLTDELPALPDPVQFGIDPESNEPLLAYPAIIEYSTDSFAIVYFSSQEEARNELNKTLARIDQLKEIKRKKEEAELLLEPTKELLKKVTEEFEEISDHSSLYRLDYSEREEIRQQLWEAKSKLTSETKQTLHNLQQIEQRLQEICLAKEERDRAKEKAKEMIKKYFSVCPLCGQDLIEGRCNNYHDLSLIDIDDILASQDSETSSKDSVVLSQLITDQGAIIAQLKVGLRRKKRSFEQGTVFLVTDDEIEGQRWLGDPFESVKFEDLGRVLTEDQLAAKEIERAKIRYQESLKYAQRQVEEGVWRLGSFVKSKNPKTGEEQWELTTQSKGLVIKYVVNRWSRQPTAPNLKYYFQIGKSLVDTKSFKLFLVDLQEPFPEDKLEESLTSTNKVKQEQVEEPDAADLEESIAKLREKWNKI

SEQ ID NO: 11 - protein, 703 aa, Thermodesulforhabdus norvegica
  tnHrpA
MKPSELRKPFPDCFNYPDDLPIIGKREEIIKTLNNHRAVIIAGATGCGKSTQLPKMCIEAGLIKKGIIGCTQPRRIAAIFLANRVSQELKTPLGQLVGFKIRFQDKTSPNTLIKYMTDGILLAEAQQDRFFRAYDVIIIDEAHERTLNIDFLLGMLQNLVAVRNDLTVVISSATIDPEKFSKAFDGAPIIEIPGKTYPIEVLYRPPENEDDEEYTYVDQAVDALEELVKKRIRGDFLIFMPTERDIRETVQRIEERTLPNMQPYPLYARMAAWQQEKIFAPTDHHKIIVATNVAETSLTIPNVKVVIDTGLARISVYSPRTGTQGLPILRISKASAEQRKGRCGRTSPGICVRLYSEDDFENMPDFTLPEIKRSNLAEVILRMISLRLGDVSTFPFIDPPSKRAISEGFATLRELGAIYEKNGEIRLTQIGYNMARLPLDPRLSRILLESLKQGAFHEVLVIVSALSIPDPRERPFGQEAMADSVHRQFADERSDFLTLLNIWRRYQAKVQEGMSRSKLKKWCKEHFLSYRRMQEWISVHDEILEIVEEFMDIPPVSQPADYEAVHKSILAGFLGRVAIHEGKGKYRGAKGREIYIFPGSYVRGTPKWIVSAEIVETSRTFARTVAEIDPAWVEEVGEHVCIRTYSNARWDFKKGNVIANERVTAFGLPIVELRPVIYGRINPQEARKIFIKQGLIDGAERLD

SEQ ID NO: 12 - protein, 1277 aa, Deltaproteobacteria bacterium
  dbHrpA
MLRDRVYVEKRLKRILKGKTQSSPAQRIIKQLKPLEKLLKESVECRSLRYSNKPEVRYPDNLPIVSKKDEIISALKTNQVVIICGETGSGKSTQIPKMCLEAGRGIAGMIGCTQPRRIAATTIAYRIAEELREELGRSVGYKIRFSDRTPQEAYIKIMTDGMLLAETHGDPGFYQYDTLIIDEAHERSVNIDFLLGLVKRLLASRPELKVIISSATLETEKFSSFFDNAPVIEVSGKVFPVEVRYRPVDLESERDGDIPYVEAALGAVEEIRREDAIGDILVFMPTEQDIIETCERLRGRLDDKENILPLFARLPGHRQKRVYTTRGPKVVVATNVAETSLTIPGIRYVVDTGLARISRYVARTRTTSLPISPISQASAEQRKGRCGRVQRGICIRLYSEEDYEKRSLYTLPEILRANLAEVILRMIYLRLGDMQSFPFVDRPNPRSVKDGLDLLVELGAIEREGEKIRLTGIGRQMARMPLDPRVSRMLLEARGMDCVGEIAVIGAALSVQDPRERPVEKASLADQARACFRDENSDFLTLLNIWNTYKTITTNSLKRKFCKDYFLSYPRMREWEGVHNQILTIFKEYSSRPYKRRQVSPTMPLYERIHRCILSGFLSNIAVKKNGGIYKGAKGKELMIFPGSSLFKKGPEWIVAAEMVKTSRLFARTVARVEPEWIEDVGGDLCKYSYSNPRWSRASGKVVASEQVSVFGLIVSKGRVVPYGPINPDEAHEIFVREALVQGNIRERFGFLEHNQDLIESLSLLEHKLRRKGIVADEESIKDFYSERLAGVYDLKGLRKRIKEAGSDEFLRMRKEDLLVEEPEEELLGRFPDSLKIDDRVFRLSYRFCPGKEEDGITVLVPSSVTSEVQPTGLDWIVPGLLNEKIRELIKALPKEYRRKLIPVAKTAEAIAKELKQVQGPLATGLSEVIQKKFDVFIPPKIWSSLKIPDHLKLRISVVDPKGKEIVSGREPGVLRKVETLSEMGTEDTDAWKVARGQWEREGLKKWDFEQLPQKVQVDESTVAYPALEPGQGCVNIKLYASLKDAMARHVEGVRVLSCLELAKELKFLKRSMKLDEEARQASIYFGGPQALEDALFERVTHILFARDVRTAKAYYEQLMAGKNALRPLSMELLEACVAVIKQYAEARQTLSSIGSNNSQNMEVLRILKEIEGDLRALVPKEFFKEYDLDTLKNLPRYLRAATVRAQRAAYDPMKDRRKRDRLEEPFRFLREMQAEIASGASEEKRKAVGEYRWMMEEFKVSLFAQELGTAYPISLN

SEQ ID NO: 13 - protein, 1255 aa, Puniceicoccales bacterium CK1056
  pbHrpA
MKGRPPLQVRYPEELPIAIHRKEIIELIQSNQVVVIAGETGSGKTTQIPKMCLDAGLAEKGKIACTQPRRVAALSISRRIAEELGVDWGAEVGAKIRFTDKTRRDTLIKVMTDGMLLTEIQGDSDLREYSVIIVDEAHERSLNIDFLLGYLKELLKRRRDLKIVITSATIDTKAFSEAFDGAPILEVSGRLYPVETIYAPIDELLEEAGEMTYVDGVVRGIELILDWNRPGDVLVFLPGEKDIREVRDMLEKRGFNHLEILPLFGRLSGQDQDRIFKSSRFRKVILSTNIAETSITIPGIRFVVDSGLARVSRYSTHTHTRRLPIEKVAQSSANQRKGRAGRLSEGVCLRLYSEQDFLSRPEFGTPEILRSNLADVILRMIAFRIGDIRTFPFIEPPAERSIRSGFELLVQLGALDKEHQLTPLGRKLAHLPADPTVGRMLLEANREGCVSELLVIAAGLSIQDPRERPMDLAKDADAMHRKFQHPESDFLTLLNIWNSYHEEMDRLSQNQLRKFCKSHFLSYLRMREWRDIHHQLERTLKEVRSFRENAEPAEYDQIHRALLSGLLSGIGQLEEANHYRATRNRKVMIFPGSGLFKKTARKSAKKKKPDAAEEKKISFKWILCAEFMETNRLYARTVARIDPNWILRIGSHVLTHKYTEPFYEEKNERVLVRERILLYGLEVATKKTAYLQVDARAATEIFIREALVEGRLLSKVPFHEANQRLLESVRDQQTRLRKGTGWALDEKLYEFYARRLERVGSYGDLRAFLRDQHGGKDDALRITENDLLQESELEKELNAFPDVADLKGLRLDLEYAYKPGEDEDGATLKIPVEEFESVEPGLIDWAVPGYICKRVEYLLRSLPKEMRKQLFPMADVSQELALKVSAEKGSLVEQLTELLWESRKVRVRKDDWSDEAVPEYLRPRVEVIDRKKKTVASGRNWQEVSQQYEQAVRSSFEKGEGREQLQIWKDGQAKFEADRVHPDSFPDLPLEIVLGDIAGLPVKAFPGLESGKNGVALKLYPDLATASRATRKGFPELCAEGLGRDLGWLERDLQKEVKRVALGFSFLMDSKALAADSLSLITRDLLAFAEPLPLQRDKVERVIAQARGKMKGLVPRYVDLLETIIGKRDKVLRLLQTSSPWEIELNALVHPKFLRELNLARLHQYPRYLEALTLRIQRARQNPAKDAEKAKPLIRFIQRYQTLKAPALEKRHLRWLLEEFKVQVFAQELGTSDKVSSKIIESAFRALEDQAGRKA

SEQ ID NO: 14 - protein, 1331 aa, Desulfobacterium vacuolatum DSM 3385
  dvHrpA
MKEIKKIEKLLNRVMCVDRPHLIRGLRGLKKKGAGNAGKRDAGEKEKQAARLYNRALRSAALRTARAKSIPRIVDFPDLPITHKKDEIIHALKHHRVVIIAGETGSGKTTQIPKFCMEAGRGAAGRIGCTQPRRIAAITVAKRLAEELREELGRSVGYKIRFDDRSSQKSIIKVMTDGILLAETQKDPFLNEYDTLIVDEAHERSLNIDFTLGILRDLVQKRRDLKLVITSATIDTEKFSKAFDGAPVIEVSGRMYPVELRYMPVQNHDDPDQDDQGYVEAAVDAVDMIHRESRQGDILMFMPTEQDITEAIELLRGRQYPGVTVLPLYARLSAHEQAKVFSRGPGRKIIVSTNVAETSLTIPGIKYVVDSGLARIPHYSPRTRTTALPVSPISRSSADQRKGRCGRVSNGVCIRLYDEADYGARALFTSPEILRSNLAEVILRMISLGLGDVASFPFIDAPASKSIKDGFDTLMELGAICTTQKRGKKSYTLTRKGRVMAGIPVDPKLSRILIEAEERGCLEEASVIASALSIADLRQRPQDKTQQADQKHALFKDPASDFITLLNIWKACHGAEKRLKSRNGLRKFCKEHYLSFKRLREWKDIHGQIMSVLREHGITGKNKISLTTGTKGLKAKEFDIGGPLYIELHKSLLCGYLANIAHKKEKHIFQAAKGQKAMIFPGSGIFNKAGNWIVAAEFVETSQLFARTAANIDPDWLEELAGPLCTRTHASPHWEKKRGEVVATEQVSLFGLVIVPERRVSYGAINPEEAGDIFIRSALVEGEVPRRFPFMDHNQELMDGLSKLEEKIRKRDILASDDEIFFFYKERLEMPFYNLKTFARYLKKRREDTFLRMTLGDLQKNQPDEDHLASLPDSLEMGMTRFDLEYGFDPGAEHDGVTLKVPAMSAGSVKNASLEYLVPGLFKEKITALIKNLPKKYRVLLMPVSTKAQIIVKEMSHRDRPLFSELSQFINRRFGVNVPASAWSDKGLEDHLKMRISIRDEKDREIAASRDKGVLKNFSDTMFPREDAFEKVCAAYEKENIVSWTLGDLPVSVPVEAAEGYTYGVYPALTREGDRVDLRLFKKQGAARASHREGVKKLYELVYESDINALKKDLKRTRKLKKYAVLVGGELSFDRALFNCVMRHLFLKEIRTRHDFESHAGDTIPQLYDIGQKLVSGVEQLCEAHDKTMETLKQIQLKNISRPQISQWVGRLESAVTALIPNGFLEIYTLERIPHLRRYVMAIGIRAQRGMVDFNRDQQKAAAVEKYTTRLNEMLNSLSVDSSREKADAIEEFFWMIEEYKVSQFAQELKTPVKISPKRLEERCRAISLMV

SEQ ID NO: 15 - protein, 1311 aa, Desulfobacter sp.
  dsHrpA
MSIKKWTAVSNGLFDIFKTLATIGGIMSISDQIKTLIPKAMCRDRYMLARALRSRQKTGQGPGKNFLKDLLSRAQASADIRQQRMDNLPQNIRFDPNLPINAEKERIIKAIQDYPVVIISGETGSGKTTQIPKFCLEAGRGVSGMIGCTQPRRIAAMTVAKRIAFELNESLGQSVGYKIRFDDHTPDNAYIKLMTDGILLAETQQDRFLNHYDTLIVDEAHERSLNIDFVLGILRSLVKNRRDLKLIITSATIDTEKFSKAFDNAPVIEVSGRMYPVELIYAPIEDDNNNGESTGAPDDQGYVEAAAGHAADLLMRTRTGDILIFMPTEQDISETMEILKGKNLSGVTILPLFARLSAGDQAKIFASGPGRKVVVSTNVAETSLTIPGIKYVVDTGLARIPAYSPRTRTTALPVSPVSQSSANQRMGRCGRVENGVCIRLFDENDFNGRPFFTTPEILRSNLAEVILRMMALGLEDVSTFPFIDPPAAKSITDGFDILLELDAIAANKPGPQTGAKKRQGKKYRLTPSGRLMARLPMDPKLSRILLNAGDTGVLKEAVIITTALTVSDIRQRPADKIQAADQKHAQFKDPASDFITLLNIWNACIDARNRLKSRSALRKWCIENFLSFKRLHEWQDIHGQITRIIKEHGIEQTAPPAEDLKAEDLESGQFEHGDPLYASIHKALLHGYLAGIAQKKEKNLFTAAKGGQAVIFPGSGLFNKAGNWIVAAEYVKTSQLFARCVGNIDPAWIEEIGQSLCTRTYSAPHWEKKRGEVVASEQVSLFGLILASGRSVAYGKINPEESGELFIRHALVQGEIYQEFGFMTHNRNLIEEIATLEDKTRQRDILASDDEIYLFYQSRLPKPFYNIRTFAKFIKDKKDDTFLRMTREDLQKTDVDEALLARFPDTLTTDQGEFALDYEFNPGAKTDGVTLKVPSQDAALISPHQVETLVPGLLREKIAALIKALPKSHRVKLMPIQQRADFIADHLPDSDAPLYSKLSGVIQKHFNLVIPASAWSDEDLADHLKMRISIRDHKDREIKSLRDLSKLGTFATQRPAQKTNAFERTKKAFEKTGLREWNFPDIEQEIQLDEGNGTRRKAFPGLCCGPDSDSVTLTLFKTREMALESHAKGVCRLFEIMFPDDIKALKKDINRTEDLRRIAPYFNDKPTFARMAYNAMAKAFFQKEIFTQKAFDDHVQALRPKLYTLGRQAMEEILTVGREYATCFDLLQSLSLASRERPLIFEALTAIFNELKNLCPANFLELYDLNRIALLPKNLECLSIRARRWVDNPAKEAQKKQLVAPYEQKLAHLIS

SEQ ID NO: 16 - protein, 742 aa, Chaetomium thermophilum var. thermophilum DSM 1495
  ctPfa1
MGASLRQSWSRSALIIPALQAPVIHSYTTSFQGACITWSEWAWLEGDAKLRHKPIAFISAGFVEPLKELKELERPESGEVTESVNDNPETNGNIDASAYPNAATPETEVLNRVTVETTVETTIRFIEQPRLNQSAVISKSVTAVGNGSSAAEEVEQVEKCEVEEITTAKETIQTDKEIQSNDGLFVFDLEGDESMLEKLTQAPPPKPPPAEKEKKTSSKPASPRASCGSDSSEEVILFKGRLAAAKGTSKRLDQSSTPEFSTFQKSSQDSKPSAEQKSSNARKTRALVVAPHNRTSQNDTLAFGMSRKKQLKGRRNSRHPPPMEEDSEEDAILADYIENMAANDEDDFFSQQLQALSGYRDLGGDHDSVNFGREDEFGLFKTGDSLGEDSGSEVSGASGTSDVETTDMLNEEKSESEEDESMAEDMDDETLAQLLAKQEEHGMGSDKLLLFNSSAAAKRDKGRQQKQHTTLPSASQVADALDNLEIGEWGAPYLRHPRKRRSKQPPNFNVSDSEVEAALRAAWQRDRERKKERKMAREALRSQGLLGKNADLNDLRVKYPHGMKLDDMKAELVSFLLSSAERLEFPPLDKHARKILHELANKFNITSKSSGSGDQRRPVFYRTKRTVRYASTKVEEATNHVDKAAMRIHRKYFHRVDIRGHKPSKLPSVTGESKARSSYKALILRDGEIVGASVPELGQDNKGRAMLEKMGWTKGMALGAADNKGILEPVAQVVKRSKAGLG

SEQ ID NO: 17 - protein, 709 aa, Thermothielavioides terrestris NRRL 8126
  ttnPfa1
MPPKWDKRPPSGRKAPRGRPTPSRGRIRQSIPSTPTMAAASHGFSMKDEARNTASHQYSLDWGSGDAKLRQKPVTFVSAGVVEPLKEQKPSSHVSESETADKRAEDAVEVTGDSARMEAAEIQEMEIIDDREGETIIEGPRQETPMIKGASTEQFVVGANESEDAQESEKKELFFFDLGEGESVLDTGLPPPRIPSPKSSLDGSDSSEEVILFKGRFAGAPGASDRTEECRPKECRPSASATASVTPLKREAEALAGPSNSESRSITRPTRPLRKRSRSRRGFRQTRRAMEDSDEDAILADYIANMTTNSDDDPLASHLRSLSGYRDLGGDDEAVNFGFDDGKSPGRNDSSDDERSSAPGYDIGNSEMDDSEMDDSVNGDDDQEMDAAVDDETLARLLAKQEELGLGGDDLLLFTSSFAQRETTKSRGKHTASASSSRAPARHASAARVADALDDLDLANWSQLTGQSRKRRSKRPPNFNVSDSKIEAALQAAWQRDRERKKIRKLEREALRAGGLLGKNMDSNDLRVKYPSGMKLDDIKAELTSFLLGSVERLDFPPLDKHARMVLHEIANKLNIKSKSTGQGNQRRPVLYRTNRTFKYASTRIEDAASHVDKAATRVHRKYFHRVDVKVQRTESPRSAGGRTSHKALTLREGEVVGASVPELGQDNKGRAMLEKMGWSKGMALGALDNKGILEPVAQVMKRSKAGLG

SEQ ID NO: 18 - protein, 700 aa, Thermothelomyces thermophilus ATCC 42464
  ttPfa1
MPPRRGRWSLPSAKASQGRLAAPRGKLPGFVPATPNAGSQSNGFSMRDEAKHTASHQAFSAWASEDAKLRQKPVTFVSAGYIEPLKERLLSEDPPGLSMPGRSSVGVIEDVGGSGQLQDATNPDDAKDIAAVPIEEETAVDIVGQISLSTEFATKSAGSLDQPSISEGGETKELFFFDLAENEPTIDPSITPPKIASPRSSSAESDSSEEIILFKGRTANSRRPLLGNENFPRATPAPPEEHDKHNSEVILSRFEKGNAQNTRPPSQVSQKRSKARRRRLQALEAMKDAEEDAILADYIANMAASSDDDLLANQIQPLTCHRDLGGDDDAIDFGVTDEKSPKGDNPLDEVEEFAESDASDTGMVDFVESEDDHDMDADTKDEALARLFAEQEELGMGSDDLLLLTSAFADTGTRKSKEKRVLKANSGRAPHEPPSATQVADAFDCLDLADWGYLSGRTRKRRSKHPPNFNVSDSEIEAALKTAWQRDRERKKSRKQERETLRSQGLLGKEAGPDDLRVKYLSGMRLDDIKLELTSFLVGSAERLEFPPLDKHARKVLHELASKFDIKSQSTGKGDQRRPVLYRTNRTVRYASTRFEDAARHVDQMASRIHRKYFHRVDVKVQKTGLTRNTGGSRSGHKALTLREGEIVGASVPELGRENKGRAMLEKMGWSKGMALGASDNQGILEPVAQVMKRSKAGLG

SEQ ID NO: 19 - protein, 718 aa, Podospora anserina
  paPfa1
MQSPTLLTFDLPPESRAMSVPFPQRRFSRVSRTQMVRFPDSALAWLQDLAHLTPTDFSLKDEVRNTQSHHLDSAWTSGTVKLRQKPVSFVSAGYSEPLKLLEDIEQDKVPPGEATESKADDMDITTVDVNLNVSAEAVIEKTTLVELDSAAKGKMVLSNSTSQDNPSSETPQEQAQDLFFFDVSGDKAIRDKHRAVHPPPLVPIRKPSLAESDSSEEVILFRGRAGNAKTVPQSNFVVRNGVATNTTTAITPTGDKTKPTAAEETSLRDDPEVIPVAREKRAGRQRSRSKASKIPKTDEDDEEDAILADYIANMSANPEDDFISDQLRSFNNRRDLGGDNFALNLGSGDENDMPVVEDLSGDEQQAESSGSGLSDADEDNGDENDEADEDDDMDADMDDEGLARLLAKQEELGLGSDELVLIPESFGVSKRGAKKGGQKRATPSSFAKSANASSVADAFDDLDLADWTVPVPRKRRSKQPPNFNISDSEIEAKLKLDWSRDRERKKERKLARESLRGQGLLDKNASPDDLRVKYPVGLRLEDFKTELVAFLISSDERLEFPPLDKHGRMVLHQLALKFNVKSQSTGKGTTRRPVLYRSKRTITFKPHQITEATRQVDGAARRVGRKYFPRADVAGPRGDTPRDGFRGSAHVSVKALVLREGEVVGASAPELGQENKGRAMLEKMGWSKGMALGALENKGILEPVAQVVKKSKAGLGRT

SEQ ID NO: 20 - protein, 657 aa, Neurospora tetrasperma FGSC 2508
  ntPfa1
MAPKKGKRPHAGPKTARFTMRDEARNTTSHQLLLGTSLRTKPVQFVSAGYIEPLKQPELLPPASPTLVGVDTAEEIQLQLNEIQEATVEAVGENSKPLGIDVQQSEPSRNDSTHDETDPVAKTDENVEATEQLFFFDVARDETVVGTDQPPVPIPNRQPLADHSDSSEEIILFRGRTTHVQPTVQPVCEPRNHATNMTRQPMVGSTGTAAASTSTKVIIAARPTSAQGGRPTSAFKRKSPKRDSKRDSKREQKYMEDDDEDEILADYIANLADDSDGDDILTSHLRTFANRRDLGGNGNSVNFGDESDDMDAMSETGGSNASDDSGENEQLDIDEEDIDDETLARLFAKQEELGMGSNELVLFSEEAAFNVQKAKNKKRAGRTEGFPSATAVADAFDGLELTDGWVNPGFIPPGRNRRNKQPPNFNVSDSEIELVLKTAWQKDRERKKQRKLEREELRAQGLLGKRANPDDLRVKYLTGMTLDDIKTELVAFLLTTEESLQFPPMDKQARKVLHELANKLKIKSQSTGKGDQRRPILYRTKATLRYKGHRSEEVVTHVDQAAVRINRKYFHRLDAKGKPSYKTPSGGGGGRSGHQAVTVREGEIVGASAPELGQENKGRAMLEKMGWSKGMGLGSLDNKGILEPVKQVVKRSKAGLG

SEQ ID NO: 21 - protein, 679 aa, Coniochaeta sp. 2T2.1
  csPfa1
MAKKPKRPAAGAGSARQKAAASQSRQRSRADFALAALREVTSPNHAFTMKDEARNTGHRSSLWGGDTRLRAKPIGFVSAGLIEPLKKDESQAAQDDAPSEGLVDDVIATDDAALQLRPDTLAVEEETSPALEVPLQSLDLSGSPTSPAPAAAPAAERSASDRSSQAASIGFVIDVKGDKKLAAQLINSTPHIPDVESIAEESDSSSEVILFKGRGNTIPSKNSVEQKRAEKTVFLDTIHYEIQSDVTKGAPDRAVPCSSARLDRQQKPDNFMDSDDEEAAIIADYIANMAEDSGDDVGEPPSRLSLLNGDLGGDTGHFGNFASESSVSSDDSAASGDDDEDENAINGDMADGHLSDSDRLASPTIDDETLARLLGKQEELGMGSDKLILASDTVGNQGSTPRGKSRRGKGVNARMQGAFASASAVADAFDDLDLMDWQRPSLQNQRKRGRRGQPPVFGLSDSEMEQNLQTAWQNDRESKKSRKIRREELRSQGLLGKHADPDDPRLRYPTGMTLEDIKSEFRAFLQGSEQRLELPPMHKSARKTLHLIARQFKVKSQSTGSGTQRRPTLIRTKYTASYTEEHLEIAMSGVGSKHFPRLDLKGKGKATQKSRGGGGNSAVTYQEGEVVGASAPELGQENKGRTMLEKMGWSIGMGLGTLDNKGILQPVAHVVKRTKAGLG

SEQ ID NO: 22 - protein, 688 aa, Monosporascus sp. GIB2
  maPfa1
MPQGKNNNKPARPQGPRPGRRKAGGLLGKILADYDGDLSSQCLADNARGHGYSLAEEARNTAYNRRGKPRLDAKLRYQPVKFISAGFMDPLKDLEVEQKALSQTQPAQKARKPNSTTAEASDEAHTPAEHLKTPEAVTEELSAPSFTLDLTGDKLLRPPQQLVTDAATPEPSCDSDSSDEVILFKGRDARRQNRTPAELSQDTSGRHDNQPDTLELREMDLELRVVEKSIQNDKISVSQETSQHHVQKTVVEAYDHIPLSTAAKRGPGRRAASASTTSDEEAAIIADYIANMQEDSDEGEDDDGEDDGPVIGTHAFHMLRDLGGTDSDAIPEEISSAEHSSDGSVDDEIDEETQKRRLELEDERMARILAKQEELGLGSDEILLYDDADSDSGEDQWQPAPKGTPRRKKKGSTKKAKIMQKKGQYPSATRMAEAFDDLDLMDWHRPSLNNFKKGPKAFDVSDSELEEAMNMAWQKDRLKKAKKKKAREELRSQGLLGKNANPDDLRVKYRGGMTIDDLANELEYFLIGTRQQLSLPPFDKQARRTIHQLANKFKIKSQSAGKGNDRYTVLYRSRATLPFEQAFFEREFARIKRTWFPRVDVDEEIVKQTRILKRAEPRKARGNHFPTYREGDVVGQHAAELGAENKGRTMLEKMGWSKGMALGTVDNKGIMVPITQVVKKNKAGLGDA

SEQ ID NO: 23 - protein, 667 aa, Hypoxylon sp. EC38
  hsPfa1
MAKNKKGGPASRFKSQRFPRRKGPLPGNPSGEYGGNNSSPGFQEFMRAHGYTLADEARNTASNRRGAFGYDAKLRYRPVTFISAGLMDPLKDLNVQLTTANEAQGSKNDTGELPATTVAPITHACSSEDYVPSSPPDEESYRNRQSVSESLTHEIQGVRPTNKSKRPPDPASGQSDDSSEEVILFKGRDRSRQDPIPARIDRNAPNTDSLELRELDIELQVVEETLHQEAARTEDYISLDNKPKGKSKQPSRQRTIQQSTTSDEDAAITADYMANIKDWEEDNEQDPEYQAAGSHAFSVLRDLGGTDSDAVPNEVSSENGTERDSEDGTDVESRRNRLEAKDERMARVLAKQEELGLGSEDILLFDGEAPDDDWLTPTKTTPRRKRKGDSKKAKIFQRKGQYPSATQMADAFDELDLMDWHRPSLHNFKKGPPAFNISDSELEEAMKSTWQKDRLKKAEKRKAREELRSQGLLGKNANPDDLRIKYLGGMSLDDLADEIEMFLLGSKEQLILPPLDKVARKTIHAIANKLKIKSQSAGAGKDRYPVLYRTKATLPFDQVTFDGVFGRVKQTWFPRVDVDDEIVNKTRIFKRTEARNGKSRFKNSLTYRDGDVVGQHAAEIGAENKGRAMLEKMGWSKGMALGTGENKGIMVPITHVVKKSKAGLGDA

SEQ ID NO: 24 - protein, 682 aa, Madurella mycetomatis
  mmPfa1
MPSRRGKRPAAGQNSARARPAAAEKNFGYWFSTNPPTRAVSDGFSMKDEARNTVFHQSKLPWGSKLRERPVTFVRAGVFEPLKDLKLFDSRDATVVEEPQEGAMENHGDNAEVDGVTAEEISVQTTEAINTVTTVKQHNPATRGLSSHSQSDAVSQPTEAQSGDTKDLFFYDLEGDHTMDGPSIAPPKISSPRSSQGASDSSEEVILYKGRSADTRAAAHKPKITHQGAPAQAAVASLSSGKKTPDATPKGPRSQNIKSTSQPHQERSKPHRSRSGRGKAVEDDEDEILADYIANMTANSDDDILTRRFQSLSSRRDLGGDDFAVHFGSADEKCPGNGDSTDNRGTGPESSDIGDSEEDDLVEIDEDEQAMDADMDDETLARLFAKQEELGIRCDELLLTSSSSFTKVGSRARAKRNRPFDELANTISVADAFDGLDIGQPVRKRRSKQPPNFNVSDSEIEAALQSAWRRDRERKKKRKMDRETLRAEGLLGKNVDPDDLRIKYPSAMTLDDFKTEITSFLLGTEERLDFPPLDKHARKVLHELASKFNIKSQSTGKGDQRRPVLYRTNRTIRYASTRVHDVNSHVEEAALRIHRKYFHRVDINGKTASPKTTAGGRGFKSLRLREGEIVGASVPELSQENKGRTMLEKMGWSKGMSLGATDNQGILEPLAQVVKHSKAGLG

SEQ ID NO: 25 - protein, 718 aa, Coniochaeta pulveracea
  cpPfa1
MAKRKKPSAGPGAARFRAAFAQGRGSRDLSSSSLREMAGLNNFTLKDEARNTGHHASAWGRASNLRAKPVSFVSAGMIEPLKEKSTFTQDDDESQEDLANTATDPKATNEDIDVAVPQVQGVEASHESESSEPPVAPDEPSLTTEPNVSETVTTTVVEDVVIDKIDELKIEPSSSMDFVIDVAGDKTLSAKLASHSAPKVPEPQFSAEDSDSSAEVILFKGRANQNRTALPAKRVTTERVVHKETIRVDVLPPQAARQPTPQPKHEPVSVAEPVIDEPSTRRTPSPTPEPDADTAGPNLDKLLASENEEDALIADYIANMVSDSGEDSEGNTRPYLMSDLGQGNPWAAKDASSNDDSDESGDDSGDDEFFNELIGADGSNAIPDSENSGEDDGMASPTIDDETMARLLAKQEELGLGSDELVLFGGQEMSTSYTVNMGKSRSRTKAEAQIIKGRRKFPSASAVADAFDELDLMDWERPSLQKPRKGGRRGKAPPDFDVSDSELELTLQTAWVKDRETKKMKKLQREELRAQGLLGKHANPDDPRLKYPTGMTLDDIKTEMRDFLLGSEPLLQLPPMDKHSRKILHELANKFKIKSQSTGSGNQRRPTLHRTKYTARYVESHFEVAISHVERKHFPRLDLKGKGKGKAPIRRGAGSSAVRYMEGEVVGASAPVIGEQNKGRNMLEKMGWSLGMGLGSVDNKGILQPVAQVVKTTKAGLG

SEQ ID NO: 26 - protein, 81 aa, Chaetomium thermophilum var. thermophilum DSM 1495
  G-Path domain
KPSKLPSVTGESKARSSYKALILRDGEIVGASVPELGQDNKGRAMLEKMGWTKGMALGAADNKGILEPVAQVVKRSKAGLG

SEQ ID NO: 27 - protein, 785 aa, Artificial Sequence
  Prp43-GP-2
TTAKQAEAVEDSDINPWTGQRHSERYFKILKARRKLPVNKQRQEFLDLYHNNQILVFVGETGSGKTTQIPQYVLYDELPHQTGKLIACTQPRRVAAMSVAQRVADELDVKLGEEVGYSIRCENKTSSKTLLKYMTDGQLLREAMHDRDMSRYSCIILDEAHERTLATDILMALLKQLSERRKDLKIIVMSATLDAQKFQSYFFNAPLLAVPGRTHPVEIFYTPEAERDYVEAAIRTVLQIHACEPEGDILLFLTGEEEIEDACRRISLEVDEMIRESDAGPMSVYPLYGTLPPHQQQRIFEKAPQPFRPGGRPGRKCIVATNIAETSLTIDGIVYVVDPGFSKQKIYNPRTRVESLLVSPISKASAQQRAGRAGRTRPGKCFRLYTEEAFKKELIEQTYPEILRSNLSNTVLELKKLGVEDLVHFDLMDPPAPETMMRALEELNYLASLDDDGELTPLGNLASEFPLDPALAVMLISSPEFYCSNEILSITSLLSVPQIWVRPANARKRADEMKAQFAHPDGDHLTLLNAYHAYKGAEARGEDMKKWCHEHFLSYRHLSSADCVRAQLKKIMETHGIELVSTPFHDKNYYTNIRRALLAGFFMQVAMRESSNSKVYKTVKDEQLVLIHPSTTVTTPYEWVVYNEFVLTTKQYVRTVTNIRPEWLLEIAPVYYDLSTFQKGEIKNALTRVAEKFRRQQAMKASKAKPSKLPSVTGESKARSSYKALILRDGEIVGASVPELGQDNKGRAMLEKMGWTKGMALGAADNKGILEPVAQVVKRSKAGLG

SEQ ID NO: 28 - DNA, 2112 bp, Artificial Sequence
  Initial nucleic acid sequences of Prp43
acaaccgcaaaacaagcagaagccgtggaagacagcgacatcaacccgtggaccggccaacgccattctgaacgttacttcaagatcctgaaggctcgtcgcaaattgccggtcaataaacagcgccaagaattcctggacctttaccacaacaaccagatactcgtctttgtgggtgaaacgggcagcggtaagactacgcagatcccgcaatatgtgctctacgatgagctgccgcaccaaaccggtaaactgattgcgtgcacccagccgcgtagagtggcggccatgtccgtggcgcagcgtgtggctgacgagctcgacgttaaactgggcgaggaagttggttattcgatccgttgcgagaacaaaacgagctccaaaaccttgctgaagtacatgaccgacggtcagctgctgcgtgaagccatgcatgatcgtgatatgtctcgctacagctgtatcattttggacgaggcgcacgagcgcaccctggcaactgacatccttatggcactgttaaagcagctgagcgagcgccgaaaagacctgaagatcatcgtgatgagcgccaccctggacgcccagaagttccagagctatttcttcaacgctccgctgctggcggttccgggtcggacccacccggtggaaattttttataccccggaagccgagcgtgattatgttgaagcagcaattcgcacggtccttcagattcacgcttgcgaaccggaaggtgatattttgttgttcttgaccggtgaagaggagatcgaggatgcctgccgtcggattagcttggaggtggacgagatgattcgtgaaagcgatgcgggccctatgagcgtttacccgctgtatggtactctgcctccgcatcagcagcaacgtatcttcgaaaaagctccgcaaccgttccgtccgggcggtcgtccgggtcgtaagtgcattgttgcgaccaatattgcggaaacctcgctaaccattgatggcatcgtttacgttgttgatccgggcttcagcaagcaaaaaatttataacccacgcacgcgcgttgagtcactattggtaagcccgatctctaaggcttcagcgcaacaacgtgcgggtcgcgcaggccgcacccgtccaggcaaatgctttcgtctgtacaccgaggaagcgtttaaaaaagaactgatcgagcagacctatccggagatcctgagatccaacctgtctaataccgtactggaacttaagaagctgggtgtcgaagacttggtgcattttgatctgatggacccgccggcaccggagacaatgatgcgtgcgcttgaggagctaaattacttggcgtctctggacgacgacggtgaactcacgccgctcggaaacctggcgagcgaattcccgctggacccggcattagcggtcatgctgattagctccccggagttctactgcagcaacgagatcctgtccatcaccagcctgttgtctgtgcctcagatttgggtgcgtccagctaatgcccgtaaacgtgcggatgagatgaaggcgcagttcgctcacccggatggtgaccacctgaccctgctcaacgcgtatcacgcgtataagggcgcggaggcccgtggcgaggacatgaagaaatggtgtcatgagcactttctgagctaccgtcacctgtcgagcgcggattgcgttcgtgcgcaactgaaaaagatcatggagacgcatggtatcgagttggtctccactccgttccacgataaaaattactacaccaatattcgccgcgctctgttggctggcttttttatgcaggttgccatgcgtgaatcttccaactccaaggtgtacaaaaccgttaaagatgagcagttggtgctgatccatccgagcacgacagtaaccactccgtatgaatgggtcgtgtacaacgaatttgttctgaccacgaaacaatatgtcagaaccgttaccaacattcgcccagagtggctgctggagatcgcaccggtttactacgacctgtcgacctttcaaaaaggcgagatcaaaaacgcgctgacccgtgttgcggaaaagttcaggcgccagcaggctatgaaggcgagcaaggcg

SEQ ID NO: 29 - DNA, 246 bp, Artificial Sequence
  Nucleic acid sequences of GP domain
aagccctcaaaactaccaagtgtaacaggagagagcaaggcgcgttctagctacaaagcgttaatcctgcgtgatggtgaaattgttggtgcgtccgtgccggaactgggccaagacaacaagggccgtgctatgctggagaaaatgggttggaccaaaggcatggcattgggcgcggcagacaataagggcatcttggagccggtggctcaggttgtcaaacgcagcaaggccggtctgggttaa

SEQ ID NO: 30 - DNA, 2358 bp, Artificial Sequence
  Initial nucleic acid sequences of Prp43-GP-2
acaaccgcaaaacaagcagaagccgtggaagacagcgacatcaacccgtggaccggccaacgccattctgaacgttacttcaagatcctgaaggctcgtcgcaaattgccggtcaataaacagcgccaagaattcctggacctttaccacaacaaccagatactcgtctttgtgggtgaaacgggcagcggtaagactacgcagatcccgcaatatgtgctctacgatgagctgccgcaccaaaccggtaaactgattgcgtgcacccagccgcgtagagtggcggccatgtccgtggcgcagcgtgtggctgacgagctcgacgttaaactgggcgaggaagttggttattcgatccgttgcgagaacaaaacgagctccaaaaccttgctgaagtacatgaccgacggtcagctgctgcgtgaagccatgcatgatcgtgatatgtctcgctacagctgtatcattttggacgaggcgcacgagcgcaccctggcaactgacatccttatggcactgttaaagcagctgagcgagcgccgaaaagacctgaagatcatcgtgatgagcgccaccctggacgcccagaagttccagagctatttcttcaacgctccgctgctggcggttccgggtcggacccacccggtggaaattttttataccccggaagccgagcgtgattatgttgaagcagcaattcgcacggtccttcagattcacgcttgcgaaccggaaggtgatattttgttgttcttgaccggtgaagaggagatcgaggatgcctgccgtcggattagcttggaggtggacgagatgattcgtgaaagcgatgcgggccctatgagcgtttacccgctgtatggtactctgcctccgcatcagcagcaacgtatcttcgaaaaagctccgcaaccgttccgtccgggcggtcgtccgggtcgtaagtgcattgttgcgaccaatattgcggaaacctcgctaaccattgatggcatcgtttacgttgttgatccgggcttcagcaagcaaaaaatttataacccacgcacgcgcgttgagtcactattggtaagcccgatctctaaggcttcagcgcaacaacgtgcgggtcgcgcaggccgcacccgtccaggcaaatgctttcgtctgtacaccgaggaagcgtttaaaaaagaactgatcgagcagacctatccggagatcctgagatccaacctgtctaataccgtactggaacttaagaagctgggtgtcgaagacttggtgcattttgatctgatggacccgccggcaccggagacaatgatgcgtgcgcttgaggagctaaattacttggcgtctctggacgacgacggtgaactcacgccgctcggaaacctggcgagcgaattcccgctggacccggcattagcggtcatgctgattagctccccggagttctactgcagcaacgagatcctgtccatcaccagcctgttgtctgtgcctcagatttgggtgcgtccagctaatgcccgtaaacgtgcggatgagatgaaggcgcagttcgctcacccggatggtgaccacctgaccctgctcaacgcgtatcacgcgtataagggcgcggaggcccgtggcgaggacatgaagaaatggtgtcatgagcactttctgagctaccgtcacctgtcgagcgcggattgcgttcgtgcgcaactgaaaaagatcatggagacgcatggtatcgagttggtctccactccgttccacgataaaaattactacaccaatattcgccgcgctctgttggctggcttttttatgcaggttgccatgcgtgaatcttccaactccaaggtgtacaaaaccgttaaagatgagcagttggtgctgatccatccgagcacgacagtaaccactccgtatgaatgggtcgtgtacaacgaatttgttctgaccacgaaacaatatgtcagaaccgttaccaacattcgcccagagtggctgctggagatcgcaccggtttactacgacctgtcgacctttcaaaaaggcgagatcaaaaacgcgctgacccgtgttgcggaaaagttcaggcgccagcaggctatgaaggcgagcaaggcgaagccctcaaaactaccaagtgtaacaggagagagcaaggcgcgttctagctacaaagcgttaatcctgcgtgatggtgaaattgttggtgcgtccgtgccggaactgggccaagacaacaagggccgtgctatgctggagaaaatgggttggaccaaaggcatggcattgggcgcggcagacaataagggcatcttggagccggtggctcaggttgtcaaacgcagcaaggccggtctgggttaa

SEQ ID NO: 31 - protein, 185 aa, Artificial Sequence
  MspA
MGLDNELSLVDGQDRTLTVQQWDTFLNGVFPLDRNRLTREWFHSGRAKYIVAGPGADEFEGTLELGYQIGFPWSLGVGINFSYTTPNILINNGNITAPPFGLNSVITPNLFPGVSISARLGNGPGIQEVATFSVRVSGAKGGVAVSNAHGTVTGAAGGVLLRPFARLIASTGDSVTTYGEPWNMN

SEQ ID NO: 32 - DNA, 40 bp, Artificial Sequence
  Region A of DNA construct X
tttttttttttttttttttttttttttttttttttttttt

SEQ ID NO: 33 - DNA, 51 bp, Artificial Sequence
  Region C of DNA construct X
tacgacgacgtttttttggtttttttctaccacgtggttactcttgcccta

SEQ ID NO: 34 - DNA, 142 bp, Artificial Sequence
  Region D of DNA construct X
tctgtctcttatacacatctcgaaacgagttctcagagcgattgacgtacagtcttagagacttagagacttagagacttagagacttagagacttagagacttagagacttagagacttagagattttaagatttttccta

SEQ ID NO: 35 - DNA, 75 bp, Artificial Sequence
  Region E of DNA construct X
tcactatcgcattctcatgatagggcaagagtaaccacgtggtagaaaaaaaccaaaaaaacgtcgtcgtatagg

SEQ ID NO: 36 - DNA, 20 bp, Artificial Sequence
  Region F of DNA construct X
tcatgagaatgcgatagtga

SEQ ID NO: 37 - RNA, 10 nt, Artificial Sequence
  Region D of RNA construct Y
uuuuuuuuuu

SEQ ID NO: 38 - RNA, 48 nt, Artificial Sequence
  Region C of RNA construct Y
ugaugaugagggauagacgaugguuguuucuguuggugcugauauugc

SEQ ID NO: 39 - DNA, 71 bp, Artificial Sequence
  Region E of RNA construct Y
tcactatcgcattctcatgatttgcaatatcagcaccaacagaaacaaccatcgtctatccctcatcatca

SEQ ID NO: 40 - DNA, 20 bp, Artificial Sequence
  Region F of RNA construct Y
tcatgagaatgcgatagtga

SEQ ID NO: 41 - DNA, 2112 bp, Artificial Sequence; identical to SEQ ID NO: 28
  Initial nucleic acid sequences of Prp43-2

SEQ ID NO: 42 - DNA, 2118 bp, Artificial Sequence
  Initial nucleic acid sequences of Prp43-3
atggctacaaccgcaaaacaagcagaagccgtggaagacagcgacatcaacccgtggaccggccaacgccattctgaacgttacttcaagatcctgaaggctcgtcgcaaattgccggtcaataaacagcgccaagaattcctggacctttaccacaacaaccagatactcgtctttgtgggtgaaacgggcagcggtaagactacgcagatcccgcaatatgtgctctacgatgagctgccgcaccaaaccggtaaactgattgcgtgcacccagccgcgtagagtggcggccatgtccgtggcgcagcgtgtggctgacgagctcgacgttaaactgggcgaggaagttggttattcgatccgttttgagaacaaaacgagctccaaaaccttgctgaagtacatgaccgacggtcagctgctgcgtgaagccatgcatgatcgtgatatgtctcgctacagctgtatcattttggacgaggcgcacgagcgcaccctggcaactgacatccttatggcactgttaaagcagctgagcgagcgccgaaaagacctgaagatcatcgtgatgagcgccaccctggacgcccagaagttccagagctatttcttcaacgctccgctgctggcggttccgggtcggacccacccggtggaaattttttataccccggaagccgagcgtgattatgttgaagcagcaattcgcacggtccttcagattcacgcttgcgaaccggaaggtgatattttgttgttcttgaccggtgaagaggagatcgaggatgcctgccgtcggattagcttggaggtggacgagatgattcgtgaaagcgatgcgggccctatgagcgtttacccgctgtatggtactctgtgcccgcatcagcagcaacgtatcttcgaaaaagctccgcaaccgttccgtccgggcggtcgtccgggtcgtaagtgcattgttgcgaccaatattgcggaaacctcgctaaccattgatggcatcgtttacgttgttgatccgggcttcagcaagcaaaaaatttataacccacgcacgcgcgttgagtcactattggtaagcccgatctctaaggcttcagcgcaacaacgtgcgggtcgcgcaggccgcacccgtccaggcaaatgctttcgtctgtacaccgaggaagcgtttaaaaaagaactgatcgagcagacctatccggagatcctgagatccaacctgtctaataccgtactggaacttaagaagctgggtgtcgaagacttggtgcattttgatctgatggacccgccggcaccggagacaatgatgcgtgcgcttgaggagctaaattacttggcgtctctggacgacgacggtgaactcacgccgctcggaaacctggcgagcgaattcccgctggacccggcattagcggtcatgctgattagctccccggagttctactgcagcaacgagatcctgtccatcaccagcctgttgtctgtgcctcagatttgggtgcgtccagctaatgcccgtaaacgtgcggatgagatgaaggcgcagttcgctcacccggatggtgaccacctgaccctgctcaacgcgtatcacgcgtataagggcgcggaggcccgtggcgaggacatgaagaaatggtgtcatgagcactttctgagctaccgtcacctgtgcagcgcggataatgttcgtgcgcaactgaaaaagatcatggagacgcatggtatcgagttggtctccactccgttccacgataaaaattactacaccaatattcgccgcgctctgttggctggcttttttatgcaggttgccatgcgtgaatcttccaactccaaggtgtacaaaaccgttaaagatgagcagttggtgctgatccatccgagcacgacagtaaccactccgtatgaatgggtcgtgtacaacgaatttgttctgaccacgaaacaatatgtcagaaccgttaccaacattcgcccagagtggctgctggagatcgcaccggtttactacgacctgtcgacctttcaaaaaggcgagatcaaaaacgcgctgacccgtgttgcggaaaagttcaggcgccagcaggctatgaaggcgagcaaggcg

SEQ ID NO: 43 - DNA, 2388 bp, Artificial Sequence
  Initial nucleic acid sequences of Prp43-GP
atggctacaaccgcaaaacaagcagaagccgtggaagacagcgacatcaacccgtggaccggccaacgccattctgaacgttacttcaagatcctgaaggctcgtcgcaaattgccggtcaataaacagcgccaagaattcctggacctttaccacaacaaccagatactcgtctttgtgggtgaaacgggcagcggtaagactacgcagatcccgcaatatgtgctctacgatgagctgccgcaccaaaccggtaaactgattgcgtgcacccagccgcgtagagtggcggccatgtccgtggcgcagcgtgtggctgacgagctcgacgttaaactgggcgaggaagttggttattcgatccgttttgagaacaaaacgagctccaaaaccttgctgaagtacatgaccgacggtcagctgctgcgtgaagccatgcatgatcgtgatatgtctcgctacagctgtatcattttggacgaggcgcacgagcgcaccctggcaactgacatccttatggcactgttaaagcagctgagcgagcgccgaaaagacctgaagatcatcgtgatgagcgccaccctggacgcccagaagttccagagctatttcttcaacgctccgctgctggcggttccgggtcggacccacccggtggaaattttttataccccggaagccgagcgtgattatgttgaagcagcaattcgcacggtccttcagattcacgcttgcgaaccggaaggtgatattttgttgttcttgaccggtgaagaggagatcgaggatgcctgccgtcggattagcttggaggtggacgagatgattcgtgaaagcgatgcgggccctatgagcgtttacccgctgtatggtactctgcctccgcatcagcagcaacgtatcttcgaaaaagctccgcaaccgttccgtccgggcggtcgtccgggtcgtaagtgcattgttgcgaccaatattgcggaaacctcgctaaccattgatggcatcgtttacgttgttgatccgggcttcagcaagcaaaaaatttataacccacgcacgcgcgttgagtcactattggtaagcccgatctctaaggcttcagcgcaacaacgtgcgggtcgcgcaggccgcacccgtccaggcaaatgctttcgtctgtacaccgaggaagcgtttaaaaaagaactgatcgagcagacctatccggagatcctgagatccaacctgtctaataccgtactggaacttaagaagctgggtgtcgaagacttggtgcattttgatctgatggacccgccggcaccggagacaatgatgcgtgcgcttgaggagctaaattacttggcgtgtctggacgacgacggtgaactcacgccgctcggaaacctggcgagcgaattcccgctggacccggcattagcggtcatgctgattagctccccggagttctactgcagcaacgagatcctgtccatcaccagcctgttgtctgtgcctcagatttgggtgcgtccagctaatgcccgtaaacgtgcggatgagatgaaggcgcagttcgctcacccggatggtgaccacctgaccctgctcaacgcgtatcacgcgtataagggcgcggaggcccgtggcgaggacatgaagaaatggtgtcatgagcactttctgagctaccgtcacctgtcgagcgcggataatgttcgtgcgcaactgaaaaagatcatggagacgcatggtatcgagttggtctccactccgttccacgataaaaattactacaccaatattcgccgcgctctgttggctggcttttttatgcaggttgccatgcgtgaatcttccaactccaaggtgtacaaaaccgttaaagatgagcagttggtgctgatccatccgagcacgacagtaaccactccgtatgaatgggtcgtgtacaacgaatttgttctgaccacgaaacaatatgtcagaaccgttaccaacattcgcccagagtggctgctggagatcgcaccggtttactacgacctgtcgacctttcaaaaaggcgagatcaaaaacgcgctgacccgtgttgcggaaaagatcaggcgccagcaggctatgaaggcgagcaaggcgtggagccatccgcaatttgaaaagaagccctcaaaactaccaagtgtaacaggagagagcaaggcgcgttctagctacaaagcgttaatcctgcgtgatggtgaaattgttggtgcgtccgtgccggaactgggccaagacaacaagggccgtgctatgctggagaaaatgggttggaccaaaggcatggcattgggcgcggcagacaataagggcatcttggagccggtggctcaggttgtcaaacgcagcaaggccggtctgggttaa

SEQ ID NO: 44 - DNA, 2388 bp, Artificial Sequence
  Initial nucleic acid sequences of Prp43-GP-3
atggctacaaccgcaaaacaagcagaagccgtggaagacagcgacatcaacccgtggaccggccaacgccattctgaacgttacttcaagatcctgaaggctcgtcgcaaattgccggtcaataaacagcgccaagaattcctggacctttaccacaacaaccagatactcgtctttgtgggtgaaacgggcagcggtaagactacgcagatcccgcaatatgtgctctacgatgagctgccgcaccaaaccggtaaactgattgcgtgcacccagccgcgtagagtggcggccatgtccgtggcgcagcgtgtggctgacgagctcgacgttaaactgggcgaggaagttggttattcgatccgttttgagaacaaaacgagctccaaaaccttgctgaagtacatgaccgacggtcagctgctgcgtgaagccatgcatgatcgtgatatgtctcgctacagctgtatcattttggacgaggcgcacgagcgcaccctggcaactgacatccttatggcactgttaaagcagctgagcgagcgccgaaaagacctgaagatcatcgtgatgagcgccaccctggacgcccagaagttccagagctatttcttcaacgctccgctgctggcggttccgggtcggacccacccggtggaaattttttataccccggaagccgagcgtgattatgttgaagcagcaattcgcacggtccttcagattcacgcttgcgaaccggaaggtgatattttgttgttcttgaccggtgaagaggagatcgaggatgcctgccgtcggattagcttggaggtggacgagatgattcgtgaaagcgatgcgggccctatgagcgtttacccgctgtatggtactctgtgcccgcatcagcagcaacgtatcttcgaaaaagctccgcaaccgttccgtccgggcggtcgtccgggtcgtaagtgcattgttgcgaccaatattgcggaaacctcgctaaccattgatggcatcgtttacgttgttgatccgggcttcagcaagcaaaaaatttataacccacgcacgcgcgttgagtcactattggtaagcccgatctctaaggcttcagcgcaacaacgtgcgggtcgcgcaggccgcacccgtccaggcaaatgctttcgtctgtacaccgaggaagcgtttaaaaaagaactgatcgagcagacctatccggagatcctgagatccaacctgtctaataccgtactggaacttaagaagctgggtgtcgaagacttggtgcattttgatctgatggacccgccggcaccggagacaatgatgcgtgcgcttgaggagctaaattacttggcgtctctggacgacgacggtgaactcacgccgctcggaaacctggcgagcgaattcccgctggacccggcattagcggtcatgctgattagctccccggagttctactgcagcaacgagatcctgtccatcaccagcctgttgtctgtgcctcagatttgggtgcgtccagctaatgcccgtaaacgtgcggatgagatgaaggcgcagttcgctcacccggatggtgaccacctgaccctgctcaacgcgtatcacgcgtataagggcgcggaggcccgtggcgaggacatgaagaaatggtgtcatgagcactttctgagctaccgtcacctgtgcagcgcggataatgttcgtgcgcaactgaaaaagatcatggagacgcatggtatcgagttggtctccactccgttccacgataaaaattactacaccaatattcgccgcgctctgttggctggcttttttatgcaggttgccatgcgtgaatcttccaactccaaggtgtacaaaaccgttaaagatgagcagttggtgctgatccatccgagcacgacagtaaccactccgtatgaatgggtcgtgtacaacgaatttgttctgaccacgaaacaatatgtcagaaccgttaccaacattcgcccagagtggctgctggagatcgcaccggtttactacgacctgtcgacctttcaaaaaggcgagatcaaaaacgcgctgacccgtgttgcggaaaagttcaggcgccagcaggctatgaaggcgagcaaggcgtggagccatccgcaatttgaaaagaagccctcaaaactaccaagtgtaacaggagagagcaaggcgcgttctagctacaaagcgttaatcctgcgtgatggtgaaattgttggtgcgtccgtgccggaactgggccaagacaacaagggccgtgctatgctggagaaaatgggttggaccaaaggcatggcattgggcgcggcagacaataagggcatcttggagccggtggctcaggttgtcaaacgcagcaaggccggtctgggttaa